European Patent Specification EP 3 589 737 B1, published October 30, 2024. Title: Haploidisierung in Sorghum. Applicant: KWS SAAT SE. The sequence listing filed with the application follows.

SEQUENCE LISTING (45 sequences)

SEQ ID NO: 1 - DNA, 2031 bp, Sorghum bicolor
acgcagtgcctatatacacaagccaccatctgtcgttgcctcctcctcctcagctcatcactagtcacacgtacacccgcaatcgattgaaaatttatcgcgttcgtccaaacaataccagagctcgacgatcatcttaattgttggatcgatctgaataatctttcttcattcgtggcctcgacgagtaagtaggtagctcatttgatcgatcaaccgcgagtgtgtgcttgatcgaaggcggcaatggcgacctactactcttcgcggcgtccatgcaacgcctgcagcacgaaggcgatggccgggagcgtggtcggcgagcccgtcgtgctggggcagagggtgacggtgctgacggtggacggcggcggcatccgtggtctcatccccggaaccatccttgccttcctcgaggcccggctgcaggagctggacgggccggaggttaggctcgcggactacttcgactacatcgccgggacgagcaccggcgggctcatcaccgccatgctcaccgcgcccggcaaggacaggcggcctctctacgctgccaaggacatcaaccaattctacatggagaattgccctcgcatcttccctcaaaagtgagtccgatcatcccggccggccgccattgttggcctcgcattattgatcgatcatgcatgcatgcatgcatgtgatgtgtaggagcagcaggcttgcggccgccatgtccgcgctgaggaagccaaggtacaacggcaagtgcctccgtaacctgatcatgagcatgctcggcgagacgagggtgagcgacacgctcaccaacgtcatcatccctaccttcgacgtcaggctgctgcagcccatcatcttctccacctacgacgtacgtacgccgccggccgccgtcgtcatgaataatcaatcagctgtacattattgcacatggctgcatgcctactgaacatgtttaatttgcaggccaagagcatgcctctgaagaacgcgctgctctccgacgtgtgcatcggcacgtccgccgcgccgacctacctcccggcgcactacttccagaccaaggacgccggcagtggcaaggaacgcgagtacaacctcatcgacggcggtgtcgccgccaacaatccggtaattaattaactgaaaacgaacgaacgcaattccatatccattgtccagaagatcgatgctaattgttgcttaggcacgtcgttgccgccggccgattgcattgcacttgcacatgcgtagacgatggttgcgatgacgcagatcaccaagaagatgcttgccagcaaggagaaggccgaggagctgtacccagtgaagccgtggaactgccgcaagttcctggtgctgtccatcgggacggggtcgacgtcggagcagggcctgtacacggcgcggcagtgctcgcggtggggcatctgccggtggatccggaacaacggcatggcccccatcatcgacatcttcatggcggcgagctcggacctggtggacatccacgtcgccgcgatgttccagtcgctccacagcgacggcgactacctgcgcatccaggacaactcgctgcacggcgccgcggccaccgtggacgcggcgacgccggagaacatgcggacgctcgtcgggatcggggagcggatgctggcgcagcgggtgtccagggtcaacgtggagacagggaggtacgaaccggtgcctggggaaggaagcaacgctgatgcgctcgctgggatcgcaaggcagctctcggaggagaggaggacaaggctcgcgcgccgcacctccgccatcgtcagctccggtggtgcctctagacgtacgtgtgcctcaaaggtctccaatgtctaagagaagtgaatttgttgcctgattaaaatcttaattaattaattctgtgggctgtggctcaaataaaactatatcattaaaaaacccgccatgaactagttctaggaaaatacgcatggttttagaaagaaaaacataaactaattctaacaaaatgtacacacctct

SEQ ID NO: 2 - DNA, 1314 bp, Artificial Sequence
  cDNA of Sorghum bicolor Phospholipase
atggcgacctactactcttcgcggcgtccatgcaacgcctgcagcacgaaggcgatggccgggagcgtggtcggcgagcccgtcgtgctggggcagagggtgacggtgctgacggtggacggcggcggcatccgtggtctcatccccggaaccatccttgccttcctcgaggcccggctgcaggagctggacgggccggaggttaggctcgcggactacttcgactacatcgccgggacgagcaccggcgggctcatcaccgccatgctcaccgcgcccggcaaggacaggcggcctctctacgctgccaaggacatcaaccaattctacatggagaattgccctcgcatcttccctcaaaagagcagcaggcttgcggccgccatgtccgcgctgaggaagccaaggtacaacggcaagtgcctccgtaacctgatcatgagcatgctcggcgagacgagggtgagcgacacgctcaccaacgtcatcatccctaccttcgacgtcaggctgctgcagcccatcatcttctccacctacgacgccaagagcatgcctctgaagaacgcgctgctctccgacgtgtgcatcggcacgtccgccgcgccgacctacctcccggcgcactacttccagaccaaggacgccggcagtggcaaggaacgcgagtacaacctcatcgacggcggtgtcgccgccaacaatccgacgatggttgcgatgacgcagatcaccaagaagatgcttgccagcaaggagaaggccgaggagctgtacccagtgaagccgtggaactgccgcaagttcctggtgctgtccatcgggacggggtcgacgtcggagcagggcctgtacacggcgcggcagtgctcgcggtggggcatctgccggtggatccggaacaacggcatggcccccatcatcgacatcttcatggcggcgagctcggacctggtggacatccacgtcgccgcgatgttccagtcgctccacagcgacggcgactacctgcgcatccaggacaactcgctgcacggcgccgcggccaccgtggacgcggcgacgccggagaacatgcggacgctcgtcgggatcggggagcggatgctggcgcagcgggtgtccagggtcaacgtggagacagggaggtacgaaccggtgcctggggaaggaagcaacgctgatgcgctcgctgggatcgcaaggcagctctcggaggagaggaggacaaggctcgcgcgccgcacctccgccatcgtcagctccggtggtgcctctagacgtacgtgtgcctcaaaggtctccaatgtctaa

SEQ ID NO: 3 - protein, 437 aa, Sorghum bicolor
MATYYSSRRPCNACSTKAMAGSVVGEPVVLGQRVTVLTVDGGGIRGLIPGTILAFLEARLQELDGPEVRLADYFDYIAGTSTGGLITAMLTAPGKDRRPLYAAKDINQFYMENCPRIFPQKSSRLAAAMSALRKPRYNGKCLRNLIMSMLGETRVSDTLTNVIIPTFDVRLLQPIIFSTYDAKSMPLKNALLSDVCIGTSAAPTYLPAHYFQTKDAGSGKEREYNLIDGGVAANNPTMVAMTQITKKMLASKEKAEELYPVKPWNCRKFLVLSIGTGSTSEQGLYTARQCSRWGICRWIRNNGMAPIIDIFMAASSDLVDIHVAAMFQSLHSDGDYLRIQDNSLHGAAATVDAATPENMRTLVGIGERMLAQRVSRVNVETGRYEPVPGEGSNADALAGIARQLSEERRTRLARRTSAIVSSGGASRRTCASKVSNV

SEQ ID NO: 4 - DNA, 2031 bp, Artificial Sequence
  genomic DNA of mutated Sorghum bicolor phospholipase R59Q
acgcagtgcctatatacacaagccaccatctgtcgttgcctcctcctcctcagctcatcactagtcacacgtacacccgcaatcgattgaaaatttatcgcgttcgtccaaacaataccagagctcgacgatcatcttaattgttggatcgatctgaataatctttcttcattcgtggcctcgacgagtaagtaggtagctcatttgatcgatcaaccgcgagtgtgtgcttgatcgaaggcggcaatggcgacctactactcttcgcggcgtccatgcaacgcctgcagcacgaaggcgatggccgggagcgtggtcggcgagcccgtcgtgctggggcagagggtgacggtgctgacggtggacggcggcggcatccgtggtctcatccccggaaccatccttgccttcctcgaggcccagctgcaggagctggacgggccggaggttaggctcgcggactacttcgactacatcgccgggacgagcaccggcgggctcatcaccgccatgctcaccgcgcccggcaaggacaggcggcctctctacgctgccaaggacatcaaccaattctacatggagaattgccctcgcatcttccctcaaaagtgagtccgatcatcccggccggccgccattgttggcctcgcattattgatcgatcatgcatgcatgcatgcatgtgatgtgtaggagcagcaggcttgcggccgccatgtccgcgctgaggaagccaaggtacaacggcaagtgcctccgtaacctgatcatgagcatgctcggcgagacgagggtgagcgacacgctcaccaacgtcatcatccctaccttcgacgtcaggctgctgcagcccatcatcttctccacctacgacgtacgtacgccgccggccgccgtcgtcatgaataatcaatcagctgtacattattgcacatggctgcatgcctactgaacatgtttaatttgcaggccaagagcatgcctctgaagaacgcgctgctctccgacgtgtgcatcggcacgtccgccgcgccgacctacctcccggcgcactacttccagaccaaggacgccggcagtggcaaggaacgcgagtacaacctcatcgacggcggtgtcgccgccaacaatccggtaattaattaactgaaaacgaacgaacgcaattccatatccattgtccagaagatcgatgctaattgttgcttaggcacgtcgttgccgccggccgattgcattgcacttgcacatgcgtagacgatggttgcgatgacgcagatcaccaagaagatgcttgccagcaaggagaaggccgaggagctgtacccagtgaagccgtggaactgccgcaagttcctggtgctgtccatcgggacggggtcgacgtcggagcagggcctgtacacggcgcggcagtgctcgcggtggggcatctgccggtggatccggaacaacggcatggcccccatcatcgacatcttcatggcggcgagctcggacctggtggacatccacgtcgccgcgatgttccagtcgctccacagcgacggcgactacctgcgcatccaggacaactcgctgcacggcgccgcggccaccgtggacgcggcgacgccggagaacatgcggacgctcgtcgggatcggggagcggatgctggcgcagcgggtgtccagggtcaacgtggagacagggaggtacgaaccggtgcctggggaaggaagcaacgctgatgcgctcgctgggatcgcaaggcagctctcggaggagaggaggacaaggctcgcgcgccgcacctccgccatcgtcagctccggtggtgcctctagacgtacgtgtgcctcaaaggtctccaatgtctaagagaagtgaatttgttgcctgattaaaatcttaattaattaattctgtgggctgtggctcaaataaaactatatcattaaaaaacccgccatgaactagttctaggaaaatacgcatggttttagaaagaaaaacataaactaattctaacaaaatgtacacacctct

SEQ ID NO: 5 - DNA, 1314 bp, Artificial Sequence
  cDNA of Sorghum bicolor phospholipase mutant R59Q
atggcgacctactactcttcgcggcgtccatgcaacgcctgcagcacgaaggcgatggccgggagcgtggtcggcgagcccgtcgtgctggggcagagggtgacggtgctgacggtggacggcggcggcatccgtggtctcatccccggaaccatccttgccttcctcgaggcccagctgcaggagctggacgggccggaggttaggctcgcggactacttcgactacatcgccgggacgagcaccggcgggctcatcaccgccatgctcaccgcgcccggcaaggacaggcggcctctctacgctgccaaggacatcaaccaattctacatggagaattgccctcgcatcttccctcaaaagagcagcaggcttgcggccgccatgtccgcgctgaggaagccaaggtacaacggcaagtgcctccgtaacctgatcatgagcatgctcggcgagacgagggtgagcgacacgctcaccaacgtcatcatccctaccttcgacgtcaggctgctgcagcccatcatcttctccacctacgacgccaagagcatgcctctgaagaacgcgctgctctccgacgtgtgcatcggcacgtccgccgcgccgacctacctcccggcgcactacttccagaccaaggacgccggcagtggcaaggaacgcgagtacaacctcatcgacggcggtgtcgccgccaacaatccgacgatggttgcgatgacgcagatcaccaagaagatgcttgccagcaaggagaaggccgaggagctgtacccagtgaagccgtggaactgccgcaagttcctggtgctgtccatcgggacggggtcgacgtcggagcagggcctgtacacggcgcggcagtgctcgcggtggggcatctgccggtggatccggaacaacggcatggcccccatcatcgacatcttcatggcggcgagctcggacctggtggacatccacgtcgccgcgatgttccagtcgctccacagcgacggcgactacctgcgcatccaggacaactcgctgcacggcgccgcggccaccgtggacgcggcgacgccggagaacatgcggacgctcgtcgggatcggggagcggatgctggcgcagcgggtgtccagggtcaacgtggagacagggaggtacgaaccggtgcctggggaaggaagcaacgctgatgcgctcgctgggatcgcaaggcagctctcggaggagaggaggacaaggctcgcgcgccgcacctccgccatcgtcagctccggtggtgcctctagacgtacgtgtgcctcaaaggtctccaatgtctaa

SEQ ID NO: 6 - protein, 437 aa, Artificial Sequence
  amino acid sequence of mutated Sorghum bicolor phospholipase R59Q
MATYYSSRRPCNACSTKAMAGSVVGEPVVLGQRVTVLTVDGGGIRGLIPGTILAFLEAQLQELDGPEVRLADYFDYIAGTSTGGLITAMLTAPGKDRRPLYAAKDINQFYMENCPRIFPQKSSRLAAAMSALRKPRYNGKCLRNLIMSMLGETRVSDTLTNVIIPTFDVRLLQPIIFSTYDAKSMPLKNALLSDVCIGTSAAPTYLPAHYFQTKDAGSGKEREYNLIDGGVAANNPTMVAMTQITKKMLASKEKAEELYPVKPWNCRKFLVLSIGTGSTSEQGLYTARQCSRWGICRWIRNNGMAPIIDIFMAASSDLVDIHVAAMFQSLHSDGDYLRIQDNSLHGAAATVDAATPENMRTLVGIGERMLAQRVSRVNVETGRYEPVPGEGSNADALAGIARQLSEERRTRLARRTSAIVSSGGASRRTCASKVSNV

SEQ ID NO: 7 - DNA, 2031 bp, Artificial Sequence
  genomic DNA of mutated Sorghum bicolor phospholipase V162I
acgcagtgcctatatacacaagccaccatctgtcgttgcctcctcctcctcagctcatcactagtcacacgtacacccgcaatcgattgaaaatttatcgcgttcgtccaaacaataccagagctcgacgatcatcttaattgttggatcgatctgaataatctttcttcattcgtggcctcgacgagtaagtaggtagctcatttgatcgatcaaccgcgagtgtgtgcttgatcgaaggcggcaatggcgacctactactcttcgcggcgtccatgcaacgcctgcagcacgaaggcgatggccgggagcgtggtcggcgagcccgtcgtgctggggcagagggtgacggtgctgacggtggacggcggcggcatccgtggtctcatccccggaaccatccttgccttcctcgaggcccggctgcaggagctggacgggccggaggttaggctcgcggactacttcgactacatcgccgggacgagcaccggcgggctcatcaccgccatgctcaccgcgcccggcaaggacaggcggcctctctacgctgccaaggacatcaaccaattctacatggagaattgccctcgcatcttccctcaaaagtgagtccgatcatcccggccggccgccattgttggcctcgcattattgatcgatcatgcatgcatgcatgcatgtgatgtgtaggagcagcaggcttgcggccgccatgtccgcgctgaggaagccaaggtacaacggcaagtgcctccgtaacctgatcatgagcatgctcggcgagacgagggtgagcgacacgctcaccaacatcatcatccctaccttcgacgtcaggctgctgcagcccatcatcttctccacctacgacgtacgtacgccgccggccgccgtcgtcatgaataatcaatcagctgtacattattgcacatggctgcatgcctactgaacatgtttaatttgcaggccaagagcatgcctctgaagaacgcgctgctctccgacgtgtgcatcggcacgtccgccgcgccgacctacctcccggcgcactacttccagaccaaggacgccggcagtggcaaggaacgcgagtacaacctcatcgacggcggtgtcgccgccaacaatccggtaattaattaactgaaaacgaacgaacgcaattccatatccattgtccagaagatcgatgctaattgttgcttaggcacgtcgttgccgccggccgattgcattgcacttgcacatgcgtagacgatggttgcgatgacgcagatcaccaagaagatgcttgccagcaaggagaaggccgaggagctgtacccagtgaagccgtggaactgccgcaagttcctggtgctgtccatcgggacggggtcgacgtcggagcagggcctgtacacggcgcggcagtgctcgcggtggggcatctgccggtggatccggaacaacggcatggcccccatcatcgacatcttcatggcggcgagctcggacctggtggacatccacgtcgccgcgatgttccagtcgctccacagcgacggcgactacctgcgcatccaggacaactcgctgcacggcgccgcggccaccgtggacgcggcgacgccggagaacatgcggacgctcgtcgggatcggggagcggatgctggcgcagcgggtgtccagggtcaacgtggagacagggaggtacgaaccggtgcctggggaaggaagcaacgctgatgcgctcgctgggatcgcaaggcagctctcggaggagaggaggacaaggctcgcgcgccgcacctccgccatcgtcagctccggtggtgcctctagacgtacgtgtgcctcaaaggtctccaatgtctaagagaagtgaatttgttgcctgattaaaatcttaattaattaattctgtgggctgtggctcaaataaaactatatcattaaaaaacccgccatgaactagttctaggaaaatacgcatggttttagaaagaaaaacataaactaattctaacaaaatgtacacacctct

SEQ ID NO: 8 - DNA, 1314 bp, Artificial Sequence
  cDNA Sorghum bicolor Phospholipase mutant V162I
atggcgacctactactcttcgcggcgtccatgcaacgcctgcagcacgaaggcgatggccgggagcgtggtcggcgagcccgtcgtgctggggcagagggtgacggtgctgacggtggacggcggcggcatccgtggtctcatccccggaaccatccttgccttcctcgaggcccggctgcaggagctggacgggccggaggttaggctcgcggactacttcgactacatcgccgggacgagcaccggcgggctcatcaccgccatgctcaccgcgcccggcaaggacaggcggcctctctacgctgccaaggacatcaaccaattctacatggagaattgccctcgcatcttccctcaaaagagcagcaggcttgcggccgccatgtccgcgctgaggaagccaaggtacaacggcaagtgcctccgtaacctgatcatgagcatgctcggcgagacgagggtgagcgacacgctcaccaacatcatcatccctaccttcgacgtcaggctgctgcagcccatcatcttctccacctacgacgccaagagcatgcctctgaagaacgcgctgctctccgacgtgtgcatcggcacgtccgccgcgccgacctacctcccggcgcactacttccagaccaaggacgccggcagtggcaaggaacgcgagtacaacctcatcgacggcggtgtcgccgccaacaatccgacgatggttgcgatgacgcagatcaccaagaagatgcttgccagcaaggagaaggccgaggagctgtacccagtgaagccgtggaactgccgcaagttcctggtgctgtccatcgggacggggtcgacgtcggagcagggcctgtacacggcgcggcagtgctcgcggtggggcatctgccggtggatccggaacaacggcatggcccccatcatcgacatcttcatggcggcgagctcggacctggtggacatccacgtcgccgcgatgttccagtcgctccacagcgacggcgactacctgcgcatccaggacaactcgctgcacggcgccgcggccaccgtggacgcggcgacgccggagaacatgcggacgctcgtcgggatcggggagcggatgctggcgcagcgggtgtccagggtcaacgtggagacagggaggtacgaaccggtgcctggggaaggaagcaacgctgatgcgctcgctgggatcgcaaggcagctctcggaggagaggaggacaaggctcgcgcgccgcacctccgccatcgtcagctccggtggtgcctctagacgtacgtgtgcctcaaaggtctccaatgtctaa

SEQ ID NO: 9 - protein, 437 aa, Artificial Sequence
  amino acid sequence of mutated Sorghum bicolor phospholipase V162I
MATYYSSRRPCNACSTKAMAGSVVGEPVVLGQRVTVLTVDGGGIRGLIPGTILAFLEARLQELDGPEVRLADYFDYIAGTSTGGLITAMLTAPGKDRRPLYAAKDINQFYMENCPRIFPQKSSRLAAAMSALRKPRYNGKCLRNLIMSMLGETRVSDTLTNIIIPTFDVRLLQPIIFSTYDAKSMPLKNALLSDVCIGTSAAPTYLPAHYFQTKDAGSGKEREYNLIDGGVAANNPTMVAMTQITKKMLASKEKAEELYPVKPWNCRKFLVLSIGTGSTSEQGLYTARQCSRWGICRWIRNNGMAPIIDIFMAASSDLVDIHVAAMFQSLHSDGDYLRIQDNSLHGAAATVDAATPENMRTLVGIGERMLAQRVSRVNVETGRYEPVPGEGSNADALAGIARQLSEERRTRLARRTSAIVSSGGASRRTCASKVSNV

SEQ ID NO: 10 - DNA, 2031 bp, Artificial Sequence
  genomic DNA of mutated Sorghum bicolor phospholipase S291L
acgcagtgcctatatacacaagccaccatctgtcgttgcctcctcctcctcagctcatcactagtcacacgtacacccgcaatcgattgaaaatttatcgcgttcgtccaaacaataccagagctcgacgatcatcttaattgttggatcgatctgaataatctttcttcattcgtggcctcgacgagtaagtaggtagctcatttgatcgatcaaccgcgagtgtgtgcttgatcgaaggcggcaatggcgacctactactcttcgcggcgtccatgcaacgcctgcagcacgaaggcgatggccgggagcgtggtcggcgagcccgtcgtgctggggcagagggtgacggtgctgacggtggacggcggcggcatccgtggtctcatccccggaaccatccttgccttcctcgaggcccggctgcaggagctggacgggccggaggttaggctcgcggactacttcgactacatcgccgggacgagcaccggcgggctcatcaccgccatgctcaccgcgcccggcaaggacaggcggcctctctacgctgccaaggacatcaaccaattctacatggagaattgccctcgcatcttccctcaaaagtgagtccgatcatcccggccggccgccattgttggcctcgcattattgatcgatcatgcatgcatgcatgcatgtgatgtgtaggagcagcaggcttgcggccgccatgtccgcgctgaggaagccaaggtacaacggcaagtgcctccgtaacctgatcatgagcatgctcggcgagacgagggtgagcgacacgctcaccaacgtcatcatccctaccttcgacgtcaggctgctgcagcccatcatcttctccacctacgacgtacgtacgccgccggccgccgtcgtcatgaataatcaatcagctgtacattattgcacatggctgcatgcctactgaacatgtttaatttgcaggccaagagcatgcctctgaagaacgcgctgctctccgacgtgtgcatcggcacgtccgccgcgccgacctacctcccggcgcactacttccagaccaaggacgccggcagtggcaaggaacgcgagtacaacctcatcgacggcggtgtcgccgccaacaatccggtaattaattaactgaaaacgaacgaacgcaattccatatccattgtccagaagatcgatgctaattgttgcttaggcacgtcgttgccgccggccgattgcattgcacttgcacatgcgtagacgatggttgcgatgacgcagatcaccaagaagatgcttgccagcaaggagaaggccgaggagctgtacccagtgaagccgtggaactgccgcaagttcctggtgctgtccatcgggacggggtcgacgtcggagcagggcctgtacacggcgcggcagtgcttgcggtggggcatctgccggtggatccggaacaacggcatggcccccatcatcgacatcttcatggcggcgagctcggacctggtggacatccacgtcgccgcgatgttccagtcgctccacagcgacggcgactacctgcgcatccaggacaactcgctgcacggcgccgcggccaccgtggacgcggcgacgccggagaacatgcggacgctcgtcgggatcggggagcggatgctggcgcagcgggtgtccagggtcaacgtggagacagggaggtacgaaccggtgcctggggaaggaagcaacgctgatgcgctcgctgggatcgcaaggcagctctcggaggagaggaggacaaggctcgcgcgccgcacctccgccatcgtcagctccggtggtgcctctagacgtacgtgtgcctcaaaggtctccaatgtctaagagaagtgaatttgttgcctgattaaaatcttaattaattaattctgtgggctgtggctcaaataaaactatatcattaaaaaacccgccatgaactagttctaggaaaatacgcatggttttagaaagaaaaacataaactaattctaacaaaatgtacacacctct

SEQ ID NO: 11 - DNA, 1314 bp, Artificial Sequence
  cDNA of Sorghum bicolor phospholipase mutant S291L
atggcgacctactactcttcgcggcgtccatgcaacgcctgcagcacgaaggcgatggccgggagcgtggtcggcgagcccgtcgtgctggggcagagggtgacggtgctgacggtggacggcggcggcatccgtggtctcatccccggaaccatccttgccttcctcgaggcccggctgcaggagctggacgggccggaggttaggctcgcggactacttcgactacatcgccgggacgagcaccggcgggctcatcaccgccatgctcaccgcgcccggcaaggacaggcggcctctctacgctgccaaggacatcaaccaattctacatggagaattgccctcgcatcttccctcaaaagagcagcaggcttgcggccgccatgtccgcgctgaggaagccaaggtacaacggcaagtgcctccgtaacctgatcatgagcatgctcggcgagacgagggtgagcgacacgctcaccaacgtcatcatccctaccttcgacgtcaggctgctgcagcccatcatcttctccacctacgacgccaagagcatgcctctgaagaacgcgctgctctccgacgtgtgcatcggcacgtccgccgcgccgacctacctcccggcgcactacttccagaccaaggacgccggcagtggcaaggaacgcgagtacaacctcatcgacggcggtgtcgccgccaacaatccgacgatggttgcgatgacgcagatcaccaagaagatgcttgccagcaaggagaaggccgaggagctgtacccagtgaagccgtggaactgccgcaagttcctggtgctgtccatcgggacggggtcgacgtcggagcagggcctgtacacggcgcggcagtgcttgcggtggggcatctgccggtggatccggaacaacggcatggcccccatcatcgacatcttcatggcggcgagctcggacctggtggacatccacgtcgccgcgatgttccagtcgctccacagcgacggcgactacctgcgcatccaggacaactcgctgcacggcgccgcggccaccgtggacgcggcgacgccggagaacatgcggacgctcgtcgggatcggggagcggatgctggcgcagcgggtgtccagggtcaacgtggagacagggaggtacgaaccggtgcctggggaaggaagcaacgctgatgcgctcgctgggatcgcaaggcagctctcggaggagaggaggacaaggctcgcgcgccgcacctccgccatcgtcagctccggtggtgcctctagacgtacgtgtgcctcaaaggtctccaatgtctaa

SEQ ID NO: 12 - protein, 437 aa, Artificial Sequence
  amino acid sequence of mutated Sorghum bicolor phospholipase S291L
MATYYSSRRPCNACSTKAMAGSVVGEPVVLGQRVTVLTVDGGGIRGLIPGTILAFLEARLQELDGPEVRLADYFDYIAGTSTGGLITAMLTAPGKDRRPLYAAKDINQFYMENCPRIFPQKSSRLAAAMSALRKPRYNGKCLRNLIMSMLGETRVSDTLTNVIIPTFDVRLLQPIIFSTYDAKSMPLKNALLSDVCIGTSAAPTYLPAHYFQTKDAGSGKEREYNLIDGGVAANNPTMVAMTQITKKMLASKEKAEELYPVKPWNCRKFLVLSIGTGSTSEQGLYTARQCLRWGICRWIRNNGMAPIIDIFMAASSDLVDIHVAAMFQSLHSDGDYLRIQDNSLHGAAATVDAATPENMRTLVGIGERMLAQRVSRVNVETGRYEPVPGEGSNADALAGIARQLSEERRTRLARRTSAIVSSGGASRRTCASKVSNV

SEQ ID NO: 13 - DNA, 2031 bp, Artificial Sequence
  genomic DNA of mutated Sorghum bicolor phospholipase Q372stop
acgcagtgcctatatacacaagccaccatctgtcgttgcctcctcctcctcagctcatcactagtcacacgtacacccgcaatcgattgaaaatttatcgcgttcgtccaaacaataccagagctcgacgatcatcttaattgttggatcgatctgaataatctttcttcattcgtggcctcgacgagtaagtaggtagctcatttgatcgatcaaccgcgagtgtgtgcttgatcgaaggcggcaatggcgacctactactcttcgcggcgtccatgcaacgcctgcagcacgaaggcgatggccgggagcgtggtcggcgagcccgtcgtgctggggcagagggtgacggtgctgacggtggacggcggcggcatccgtggtctcatccccggaaccatccttgccttcctcgaggcccggctgcaggagctggacgggccggaggttaggctcgcggactacttcgactacatcgccgggacgagcaccggcgggctcatcaccgccatgctcaccgcgcccggcaaggacaggcggcctctctacgctgccaaggacatcaaccaattctacatggagaattgccctcgcatcttccctcaaaagtgagtccgatcatcccggccggccgccattgttggcctcgcattattgatcgatcatgcatgcatgcatgcatgtgatgtgtaggagcagcaggcttgcggccgccatgtccgcgctgaggaagccaaggtacaacggcaagtgcctccgtaacctgatcatgagcatgctcggcgagacgagggtgagcgacacgctcaccaacgtcatcatccctaccttcgacgtcaggctgctgcagcccatcatcttctccacctacgacgtacgtacgccgccggccgccgtcgtcatgaataatcaatcagctgtacattattgcacatggctgcatgcctactgaacatgtttaatttgcaggccaagagcatgcctctgaagaacgcgctgctctccgacgtgtgcatcggcacgtccgccgcgccgacctacctcccggcgcactacttccagaccaaggacgccggcagtggcaaggaacgcgagtacaacctcatcgacggcggtgtcgccgccaacaatccggtaattaattaactgaaaacgaacgaacgcaattccatatccattgtccagaagatcgatgctaattgttgcttaggcacgtcgttgccgccggccgattgcattgcacttgcacatgcgtagacgatggttgcgatgacgcagatcaccaagaagatgcttgccagcaaggagaaggccgaggagctgtacccagtgaagccgtggaactgccgcaagttcctggtgctgtccatcgggacggggtcgacgtcggagcagggcctgtacacggcgcggcagtgctcgcggtggggcatctgccggtggatccggaacaacggcatggcccccatcatcgacatcttcatggcggcgagctcggacctggtggacatccacgtcgccgcgatgttccagtcgctccacagcgacggcgactacctgcgcatccaggacaactcgctgcacggcgccgcggccaccgtggacgcggcgacgccggagaacatgcggacgctcgtcgggatcggggagcggatgctggcgtagcgggtgtccagggtcaacgtggagacagggaggtacgaaccggtgcctggggaaggaagcaacgctgatgcgctcgctgggatcgcaaggcagctctcggaggagaggaggacaaggctcgcgcgccgcacctccgccatcgtcagctccggtggtgcctctagacgtacgtgtgcctcaaaggtctccaatgtctaagagaagtgaatttgttgcctgattaaaatcttaattaattaattctgtgggctgtggctcaaataaaactatatcattaaaaaacccgccatgaactagttctaggaaaatacgcatggttttagaaagaaaaacataaactaattctaacaaaatgtacacacctct

SEQ ID NO: 14 - DNA, 1116 bp, Artificial Sequence
  cDNA of Sorghum bicolor phospholipase mutant Q372stop
atggcgacctactactcttcgcggcgtccatgcaacgcctgcagcacgaaggcgatggccgggagcgtggtcggcgagcccgtcgtgctggggcagagggtgacggtgctgacggtggacggcggcggcatccgtggtctcatccccggaaccatccttgccttcctcgaggcccggctgcaggagctggacgggccggaggttaggctcgcggactacttcgactacatcgccgggacgagcaccggcgggctcatcaccgccatgctcaccgcgcccggcaaggacaggcggcctctctacgctgccaaggacatcaaccaattctacatggagaattgccctcgcatcttccctcaaaagagcagcaggcttgcggccgccatgtccgcgctgaggaagccaaggtacaacggcaagtgcctccgtaacctgatcatgagcatgctcggcgagacgagggtgagcgacacgctcaccaacgtcatcatccctaccttcgacgtcaggctgctgcagcccatcatcttctccacctacgacgccaagagcatgcctctgaagaacgcgctgctctccgacgtgtgcatcggcacgtccgccgcgccgacctacctcccggcgcactacttccagaccaaggacgccggcagtggcaaggaacgcgagtacaacctcatcgacggcggtgtcgccgccaacaatccgacgatggttgcgatgacgcagatcaccaagaagatgcttgccagcaaggagaaggccgaggagctgtacccagtgaagccgtggaactgccgcaagttcctggtgctgtccatcgggacggggtcgacgtcggagcagggcctgtacacggcgcggcagtgctcgcggtggggcatctgccggtggatccggaacaacggcatggcccccatcatcgacatcttcatggcggcgagctcggacctggtggacatccacgtcgccgcgatgttccagtcgctccacagcgacggcgactacctgcgcatccaggacaactcgctgcacggcgccgcggccaccgtggacgcggcgacgccggagaacatgcggacgctcgtcgggatcggggagcggatgctggcgtag

SEQ ID NO: 15 - protein, 371 aa, Artificial Sequence
  amino acid sequence of mutated Sorghum bicolor phospholipase Q372stop
MATYYSSRRPCNACSTKAMAGSVVGEPVVLGQRVTVLTVDGGGIRGLIPGTILAFLEARLQELDGPEVRLADYFDYIAGTSTGGLITAMLTAPGKDRRPLYAAKDINQFYMENCPRIFPQKSSRLAAAMSALRKPRYNGKCLRNLIMSMLGETRVSDTLTNVIIPTFDVRLLQPIIFSTYDAKSMPLKNALLSDVCIGTSAAPTYLPAHYFQTKDAGSGKEREYNLIDGGVAANNPTMVAMTQITKKMLASKEKAEELYPVKPWNCRKFLVLSIGTGSTSEQGLYTARQCSRWGICRWIRNNGMAPIIDIFMAASSDLVDIHVAAMFQSLHSDGDYLRIQDNSLHGAAATVDAATPENMRTLVGIGERMLA

SEQ ID NO: 16 - DNA, 2979 bp, Helianthus annuus
atgaataacatcaatcttgtaatagtttcgcttgtaatcgcgattgtagccatccaaccccttgcgcaagagcaaaccgatgtaggtgaggcaaatttcgtcactgttcttagcatcgatggtgggggtgttcgtggcattgttcccgccaccttgcttgcttttcttgaatccaaaattcaggtactcgaacttaaaatgcacatgtgcatcatattacaagctgtaacttattattgaaatgtgccgtctcttcggataggaaatagatgggccagatgcacgaattgcggattattttgatgtaatagccggaacaagcacaggagggctgatgacaactatgcttgcagctcctaatgagaaaaatcgtcccatgttcgccgcaaaagacattaccaacttctactttcaacattcgcctaggatcttccctaaaatagggtaaactctaactagtttccggatctataagatcatcattaaatacaagtttcattttctttttcgaatcaaatacagacacacatttgatgaggcgcaaccttatccttctcaaaacgaagcctgcgaaatggggtattctcctacaaagacttttgtaattcatgttctagtgggtgtttggatgtgcgttttaaaactgattattatttacatgtagtttctgaagaaaataaaacagttattcaaacactttttgttaataattctactagaaaaaaaaaatccttgtcaggaaattaattaaaaaaaagttaccatctattaaagttctttcttactaatcaaaagtttttaaattttattatcatgttattataactaaacatacacatccaaacactatctcataccacatgattacacaagtctattatttgaatatgctaacttagtattttcatataataagtttttaaaacgccacatccaaaacccttgattcttattttacattgtgtagctaaaacagtgtttatacataaaaacaatcagttatataaatcaaagcattatttaactaaagtaagctcggttcaaactcgataagagaattaatatatacgagtcgagttcctgttgaccagatttcgctagtgttaagtttcgagttcaaaattgtatatgaacttgaacctgtgtatcatcatacttgacatttaaaccataatgttgttgaataaataaagtgattttattttgtagtcggaccaaattcatgaattcggtagtaaccgtacttggtgaggccaccggaccaaagtatgatggtaaatatcttcgagccatggcaaagatgatgttaaaaaacctcactattaaagatacgttgacgaatgttgtcatacctgctttcgacattaggcggcttcaacctgttatcttctcctctgctcaagtaattaaactcgttttttatatttatagcagttctctatttaaaattgattgtgtatcataaaatggtttctgtttgatacgtttagggaaaagaggtcgcgtggaaaaatgctttgctagcagacgtatgcattagtaccgcggcggcaccaacatttttcccgccatactattttgagactagagacgtcgatggaaccaagcacacttttgatctaatcgatggcggggtagctgcaaacaatccggtagttacatttcaacaatattgagtttgcattttatttttaggacaagtagtcacattagggtgaagggtgtgttcaagctcatcccgaaggtgggagcggtgttcccactcgtacctcatggcgcattttcttctttgttgcagctccaattttaaaaagccaccccgccttttccattccatagcgccacgtcaactgggaaatggtgttcccactggtattggagatttggaggcgctacgccacctctgtcatcccgaagccacaccctccacccttaggagtgttatcggttcagttttcggtttatacagtttaaaggtttttttttggttgaaaccaaaaaccgaactgaactgaacggaattcgggtagttcacaactgaaccaaaaactgaatccatattcggttttctgtttgaccgaataatcattatttgttatttgattgtgcgaggttaaataagattgagcaaaaattgtaattaattggatttggctaaatgacaatttaaataaccgttatttgttatccgattcaaaccgaacacccaactcgatttggtttaataccgaaccgacaaccggatacgtaattcagttcgctattaaaaggttcgggtttggtagggtttaacccatttgaaatcgaatcttcagagaaagggttcgctaatgtcacccacataaccaaagaaatcttgtttaaatgttaatggcagacacatttggctatcacacatataaccaaagaagcggtgatggggaaatacaggttctctggcccggaggttttcgacggaagacggatgcttgtgctttcactcggcactggtacgcagacgtacaatgacttatatactgcacaaaaggctgcaaaatgggggttgcttagttggatctttaccaatggtactgcgccaatcctccgcatttttggtgatgccatgtcagatatggtcgacatccatgtgtcaactatattccaatcgttgcaagtcgaaaaaaactatctgcgtattcaggtataactaagaacatataaatataatgttgtataggttacatgtttagtaacaaggagtttttttatgggcaggaagataacttgaaaggggaagcaactgcaatggatatttcatcacctgagaacatgagggcgctagaggacattggcaagaaattgttgaagaaaccgttgtcgagattggatgtggagacaggcaagcttgaaccagttaaaggagaaggtacgaatgctgatgcattagcacgtttcgccactttgctttgtgccgaacgaaagcgccgcaatccagcttaa

SEQ ID NO: 17 - DNA, 1305 bp, Artificial Sequence
  cDNA of Helianthus annuus phospholipase
atgaataacatcaatcttgtaatagtttcgcttgtaatcgcgattgtagccatccaaccccttgcgcaagagcaaaccgatgtaggtgaggcaaatttcgtcactgttcttagcatcgatggtgggggtgttcgtggcattgttcccgccaccttgcttgcttttcttgaatccaaaattcaggaaatagatgggccagatgcacgaattgcggattattttgatgtaatagccggaacaagcacaggagggctgatgacaactatgcttgcagctcctaatgagaaaaatcgtcccatgttcgccgcaaaagacattaccaacttctactttcaacattcgcctaggatcttccctaaaataggacacacatttgatgaggcgcaaccttatccttctcaaaacgaagcctgcgaaatgggtcggaccaaattcatgaattcggtagtaaccgtacttggtgaggccaccggaccaaagtatgatggtaaatatcttcgagccatggcaaagatgatgttaaaaaacctcactattaaagatacgttgacgaatattgtcatacctgctttcgacatcaggcggcttcaacctgttatcttctcctctgctcaaggaaaagaggtcgcgtggaaaaatgctttgctagcagacgtatgcattagtaccgcggcggcaccaacgtttttcccgccatactattttgagactagagatgtcgatggaaccaagcacacttttgatctaatcgatggcggggtagctgcaaacaatccgacacatttggctatcacacatataaccaaagaagcggtgatggggaaatacaggttctctggcccggaggttttcgacggcagacggatgcttgtgctttcactcggcactggtacgcagacgtacaatgacttatacactgcacaaaaggctgcaaaatgggggttgcttagttggatctttaccaatggtactgcgccaatcctccgcatttttggtgatgccatgtcagatatggtcgacatccatgtgtcaactatattccaatcgttgcaagtcgaaaaaaactatctgcgtattcaggaagataacttgaaaggggaagcaactgcaatggatatttcatcacccgagaacatgagggcgctagaggacattggcaagaaattgttgaagaaaccgttgtcgagattggatgtggagacaggcaagcttgaaccagttaaaggagaaggtacgaatgctgatgcattagcacgtttcgccactttgctttgtgccgaacgaaagcgccgcaatccagcttaa

SEQ ID NO: 18 - protein, 434 aa, Helianthus annuus
MNNINLVIVSLVIAIVAIQPLAQEQTDVGEANFVTVLSIDGGGVRGIVPATLLAFLESKIQEIDGPDARIADYFDVIAGTSTGGLMTTMLAAPNEKNRPMFAAKDITNFYFQHSPRIFPKIGHTFDEAQPYPSQNEACEMGRTKFMNSVVTVLGEATGPKYDGKYLRAMAKMMLKNLTIKDTLTNIVIPAFDIRRLQPVIFSSAQGKEVAWKNALLADVCISTAAAPTFFPPYYFETRDVDGTKHTFDLIDGGVAANNPTHLAITHITKEAVMGKYRFSGPEVFDGRRMLVLSLGTGTQTYNDLYTAQKAAKWGLLSWIFTNGTAPILRIFGDAMSDMVDIHVSTIFQSLQVEKNYLRIQEDNLKGEATAMDISSPENMRALEDIGKKLLKKPLSRLDVETGKLEPVKGEGTNADALARFATLLCAERKRRNPA

SEQ ID NO: 19 - DNA, 1531 bp, Hordeum vulgare
atggcaagctactggtgccggcgaccgtgcgagtcgtgcagcacgagggcgatggcgggcagcgtggtcggccagccggtggcgccggggcagagggtgacggtgctgaccatcgacggcggcggcatccgcggcctcatcccgggcaccatcctcgccttcctcgaggccaggctgcaggagctggacgggccggacgcgcgcctggccgactacttcgactgcatcgccggcaccagcaccggcgggctcatcaccgccatgctcaccgcgcccggccaggacggccgcccgctcttcgccgccaaggacgtcaaccgcttctacctcgacaacgggccctacatcttcccccaaaggcgagagcacgagcgatctcatggccatggatcatgccagctgaaccggtgattgatgtgtgaattgtgttgagctgtgccaggaggtgcgcgctcgccgcggtgaccgcgtcgctgaggcggccgaggtacagcggcaagtacctgcacggcaagatcaggagcatgctgggcgagacgaggctgtgcgacgcgctcaccgacgtcgtcatccccaccttcgacgtcaagcttctccagcccatcatcttctccacatacgacgtatgctaatttacgccattgatcagatagatccatcctccttggatcagacagacatggggctaaaatcgttgaaggatcatgcgtgcaggccaggaacatgcccctgaagaacgcgcggcttgccgacatctgcatcggcacctccgccgccccgacctacctcccggcgcaccacttccacacccaagacgacaacggtaaggagcgcgagtacaacctcatcgacggcggcgtcgccgccaacaatccggtaaccaaccaatcaagcgtccatcagtcatcacatattcagatacgctgcccgagcacactgatgaactgagttgtgagagatgcagacgatggtgaccatgacgcagatcaccaagaagatgatggtcaaggacagggaggagctgtacccggtgaagccgtcggactgcggcaagttcctggtgctgtccatcgggaccggctcgacgtcggaccaggggctgtacacggccaagcagtgctcccagtggggcatcatccgctggctgcgcaacaagggcatggcgcccatcatcgacatcttcatggcggccagctccgacctcgtcgacatccacgccgccgtgctcttccagtcgctgcacagcgacggtaactacctccgcatccaggacaactcgctccacggcccagccgcgacggtggacgccgccacgcccgagaacatggcggagctcctcaggatcggcgagcggatgttggcacagagggtgtccagggtgaacgtcgagaccgggaggtacgaggagatacggggcgccgggagcaacgccgacgcgctcgccggcttcgccaaacagctctccgacgagaggaggacaaggctcggccgccggcgcgttggcgccggccgtctgaaatccagacgctga

SEQ ID NO: 20 - DNA, 1269 bp, Artificial Sequence
  cDNA of Hordeum vulgare phospholipase
atggcaagctactggtgccggcgaccgtgcgagtcgtgcagcacgagggcgatggcgggcagcgtggtcggccagccggtggcgccggggcagagggtgacggtgctgaccatcgacggcggcggcatccgcggcctcatcccgggcaccatcctcgccttcctcgaggccaggctgcaggagctggacgggccggacgcgcgcctggccgactacttcgactgcatcgccggcaccagcaccggcgggctcatcaccgccatgctcaccgcgcccggccaggacggccgcccgctcttcgccgccaaggacgtcaaccgcttctacctcgacaacgggccctacatcttcccccaaaggaggtgcgcgctcgccgcggtgaccgcgtcgctgaggcggccgaggtacagcggcaagtacctgcacggcaagatcaggagcatgctgggcgagacgaggctgtgcgacgcgctcaccgacgtcgtcatccccaccttcgacgtcaagcttctccagcccatcatcttctccacatacgacgccaggaacatgcccctgaagaacgcgcggcttgccgacatctgcatcggcacctccgccgccccgacctacctcccggcgcaccacttccacacccaagacgacaacggtaaggagcgcgagtacaacctcatcgacggcggcgtcgccgccaacaatccgacgatggtgaccatgacgcagatcaccaagaagatgatggtcaaggacagggaggagctgtacccggtgaagccgtcggactgcggcaagttcctggtgctgtccatcgggaccggctcgacgtcggaccaggggctgtacacggccaagcagtgctcccagtggggcatcatccgctggctgcgcaacaagggcatggcgcccatcatcgacatcttcatggcggccagctccgacctcgtcgacatccacgccgccgtgctcttccagtcgctgcacagcgacggtaactacctccgcatccaggacaactcgctccacggcccagccgcgacggtggacgccgccacgcccgagaacatggcggagctcctcaggatcggcgagcggatgttggcacagagggtgtccagggtgaacgtcgagaccgggaggtacgaggagatacggggcgccgggagcaacgccgacgcgctcgccggcttcgccaaacagctctccgacgagaggaggacaaggctcggccgccggcgcgttggcgccggccgtctgaaatccagacgctga

SEQ ID NO: 21 - protein, 422 aa, Hordeum vulgare
MASYWCRRPCESCSTRAMAGSVVGQPVAPGQRVTVLTIDGGGIRGLIPGTILAFLEARLQELDGPDARLADYFDCIAGTSTGGLITAMLTAPGQDGRPLFAAKDVNRFYLDNGPYIFPQRRCALAAVTASLRRPRYSGKYLHGKIRSMLGETRLCDALTDVVIPTFDVKLLQPIIFSTYDARNMPLKNARLADICIGTSAAPTYLPAHHFHTQDDNGKEREYNLIDGGVAANNPTMVTMTQITKKMMVKDREELYPVKPSDCGKFLVLSIGTGSTSDQGLYTAKQCSQWGIIRWLRNKGMAPIIDIFMAASSDLVDIHAAVLFQSLHSDGNYLRIQDNSLHGPAATVDAATPENMAELLRIGERMLAQRVSRVNVETGRYEEIRGAGSNADALAGFAKQLSDERRTRLGRRRVGAGRLKSRR

SEQ ID NO: 22 - DNA, 9001 bp, Beta vulgaris
  misc_feature (2702)..(2702): n is a, c, g, or t
ttttccaacaacataccgagtagttttctccaagtttaagttatttatgttattgtaattgtaatgtaagagctagtaaagctcagtttagtttctttgtttttagtatgaatgtaccatttttagtatgtaattatgcttttaattaatgcaaaattttccgttgtaaaaaaaagtctacatgtccctcttgcagagataaatgtaagggacattattgcttagttctcgactaatttacaataagtttataattggttatcatggttcatgagtactcctgttcatagaaggacaataatttataaaggtttcttagtagcttccaatgacggagctcaatgaccctgttaattagctaagtaataagttggccattagccaataacaactgtattattagctagtaagttcattagatcgatataacttataagtctaatgaatataaatatgaataagatggaactgaaatgagttttatatttgaaaaattagtggcatacgtgcttaaacgtttttttgattatggctagaagacttagaacgaagttggaggaattcttcattcatataaatttatgctagataaactaatagccagtcaagtcaagtttatgtttttaaaaaaaatcttatctcatgtagtacgagaatctttattttataatttcgttataataaatatgcatttcactcctttcaaatcgttagctacatcacttctgcaaccaagcaagcaagccataatatttaatcacaggttctttaatactatagtctatatatacatgcaatccacttacattaattatcatcttattctcccatcatcaagaaaacacattacaatccaaagaaataaaacatggagaattctagatctctgggtaaccctgttagccctagaccccctaatcatggtaatctcataacaattttaagtattgatgggggaggcattaggggaataatccctgcagttatgcttgaattccttgaatcacaactccaggtatgtacataattaagaaatgatgatatacgatcatctttagtactcttgttaaatgatttgacgtaagaaatcatgtatatattatgcatgccttactataatattgcgtgcatgttcataatcacaacagaagttagatggtgaggaagcaagattggctgattattttgatgttattgccggaacgagcaccggtggcctcataactgccatgttaaccgcccctaacgacaaaactcggccactctacgccgccaaggagattactcctttttatcttgagcattgtccgaagatcttccgccaaccaaggtaaataaatcaaatttatcatctatgtatatcaggattggtaaattagagaggatgaaaaacccttaaatgcttggaactattaacgctcgagttccaattatgggccattgtctcttataggtctcaactattgatttttttctatagcaggcgcggatgtaagattttgaatttggaagggtcctaactaaaccaaagaaataaattacaatgaccatattaacatataagaagtttagttttaacaataagaaaaccaacagttggtcttgtaagagaccgtctacttttaatttaaaagtaggcgcggcccaagcccaatattaagaagagaatagatcatatttcttaatatagtgactactttaatctatttagtgaccattttaatctatttagtgaccagtttaatctattcattaataacattctttaattcatttagtgactgatttaatccatttagtgactagcttaatccattttgtaagactgacggactatttttaaaaattgtttgttctaattcaaaatttagaagggaaataaaagaaggagaagagaatggacgactaggatggtgcaagatacctaaaaaaagtgttaggttagagagaaattgaatgggcttcttaggagaatgtaggtttgcattgtctaattttatattaaaattagaccgtctattataataatttgtggaaaacaaaactttatattatttgaatcatgtattagatataccttaattatattgatatcttaatgttatcttcatttttagtaaattcaacagatttgatttgtacatccgttaacatatgcgacactaacatttgatatcttcagttatatgttcataatttttttttttaaaaagttggacataaatttggtaaacgaaaatagagacaaattcacaattttacatagtaatattattttcaagtatttggaaacaagcttggtcaaacttaatatagcaataccgtagaaagtcaaattattgaatttatttgaaacaaaaggagaataatcgttatatcacaaaaaaaaaagtattaaaattagagctaaattaagagagattggtagcattcaagataatgaaatgatgattagatataaaaaagaaaagatgataaaagagaaaagttaaagaacaggaagggcatgttctcttcagcataaaacagctgaactgaactaacctgaattgaactgattggagctgaactgaactgaactgaactgaactgaattgaatttaatttaatttaattgtattgaattaaattaaatttaatttaatttaattgaattgaattaaattgaatgtaataaatatataaataatatttaaacaatnagtacagttattataataataattgtgcccttctgaaattgttaaggcacgtcgtttgcaagatttgtccttttgcattaaaatttgggtgcaaatcctgcacaaattgaaatatatagtattatctctccactcatttttatcttcttgtatcattttaggctcgacaataatgactctgccagaggggtagttgaaccttcttatatcatcatcataattcataataataattttattatatatactccctccgttccaaaatatagttctcgtttcttttttttacgatgatttgtgcaagtagaatctaagtggaataataaaatttttttgtttatttaaataaatattgtatggaaaaggatgattttaggagagaaaaatggaaaataattggtgaaagagtattaattgtaatattttagttgaataaataacagaaaaaccaaaatataagaagcaaataaatgatgggacacgatctttgtagacaaattacagaaaaatttggaaacgaatatggaaatgggaactatattttgggacacccaaatagaaatgggaactatattttgggacggagggagtaatattaataatcataaattattaataataatagtaataattaatgatactaatgataattaataaccgaagatcgcgtgattatttgtgttggagttgtagtgggatatttggttcaatagggactctaatgaagctgctaagcgggccgaaatacgatggaaagtaccttcacaatctagtaaaggaattgctcggacaaagaaggttgcatcaagcgttgactaatgtggttatcccaacttttgatatcaagaatcttcagcctgttctcttttctacttatatggtatgttgttgaatttccaatttattgaagtacattattattgtacccttggttatcttattcattagcaaatactagcattcaaatagcatttatagtgatttgtcaagaaaaaaaataagtagaggaatcatagttatcacttattagaactacctcttttagaagaatatacttcctctatttttttagatggaacatttacctttttggtgagtagattaaaataatcatatgttgtatttaaaaaaacagaattagtatatatcttcttttgtgtcatataatacacttgatcaatttaaaagataacatgattccaatattgacttttttatacacataatttcacatgtcaaataatagaaaaaaagtcaactttgctgaatttggagatgataatacatagtttatgtgttggttaagtaatttcatactactacattgatagattatgaaattgatcaagaaaactaatcaataattaatgattataatgatctaggtcccaattgctaaagaattggacgtgttgctgtcagacatatgcataggcacgtctgcagctccaacgttcctaccagcgcatcattttgaaaacaaagatgatcagggcaatgtcaaagaattcaacctcattgatggtggtattgctgccaataatcctgtaagattatttcttcatccatgtttggattttctctccatccctaaatttaatttgattaggaattagtcattcttaataaaaattatgaatcatcaattaaattatctaataaaaagtaattcaaacatttgttcgatataatgtacttattttttttattaaattttaattttcagacatattccaaatgtcgtcctacaaaagaaattgcaaatccatctaaaaacttcgtttgatacatctaataatgtatgttcgagtcaatcattaaattttcatatcaagataaatatcaaagtaagatgtttcaaacttttacttagtcgattaattctattaattccagtcaatttaccatcaacttcttcggtcttcccaaaacaaatggaaaaatatatattcactgcatacgtgtctttgtgttatattcctatctctaaagtatttaagtttttatgatattaggacatatatattctctagtatttaatgagaaagatcgaaaagttttcgtatattcataaaaccttaacaactgctattcaaaatatacgataagtttcatcaacattacccactaattaaatgtaatttcactgtataagtacagtcattagtggcaataagcgaagtgacaaaacaaatagtgaagagcaacccgaatttcttcccgataaaggccacggatcgtgaacggttgctggtgatatcgttagggactggatccgacaaggtagagcagctctataatgctaaaagcgcagcaaagtggggaattatttcatggttatttgacaatggtaatactccactacttgatgcttttaatcaatcaaaggctgatatggtcgatttccacaattctgtggcctttcaagcatatggttctcttgacaattatcttcgcatccaagtaagttatttttattatacggatttggatgtttatgtacgtatatatacttctgttaaaggttgataagatgagagttacgcgctcattttaccaaggatctttggtttcaatggtaatttgggaccggtcagacccgtggctgcgggcctatcacggtcaagaatttttatttcaggctcgcaccgtcacgagcctgcctagatggctcgcgagccgaacactcatttcctttgctttttagcctaaaactgtcaaaagtccaaaaaacgacataaaacacgggccagctcgcaggagccacgagcccagtccgtggataaaatcttgaaatttcaggcccgacccaccatttccccaaacccgcgggccgagcccgtgaacaagctcatgccctgatgcccaggtctaggtctgcctcgcacggagccttcatcccgaagcccattacaagccagacacccaactccctacaacaccacatcaacccttccaatccactcgccttccctcttcactgctgccggctgccctctaggtttatcattttttctaagctcttttgtctaagttaaatccactggtttctttcattttctttttgatttaagttcgattaccaatgtttctttaactttgcaacttttggggagataccttattgtaatttgctctaatgaaagtttcttatgcttataataatgctcaattgtctttcttgatctagtaatctgagagttatccagttttaaatagttagagctagtttcactaatggtggcaataagggtgtggcagggggcgatgcttggttttggactttggtaatggtggtaatgaagggaggttacacagtgaggatggtggttggtgtaattggtggggaaactcggggtagagagataacccctaaaggcgagattatgcttagtcaatcgaaaggtgtgcctattttaagcggaccacctaaaggtcggattattataatcaatttttcctaaataaattgcaatttgtggttggatttctagtttgaaactaaatctcaattgcaagtctgcaaccgtatgaactatgaaccattttgaggttaatatatctatagatttttatttcaaaaaaatataaaaatatattatttcaaaaaggtccaagaatacgtcttttaagagtgtccaagaacatctaaccacgagttatatatttgtctattatgtggtgatcactttttcaagatttgaggtctttaattaggccttgatgatatagatttgttagagaaaaacatttgcttgattaaaaaaggaaataaatgatatgacaaatgactaattgactcatgtctaaccttttaaatgtggtgtgatttaactcgacatttaatatgtggttggtttgataaattttagcgagcacgctttatataagtgtaacttatatatcttgtgcataagtttagttatttattttttactttattaaacaaaattgataaatatgatatagttaattaaatatattactctcataaatcaagctaccctaaatctgtaaatgcaaattatattgcaggatgatacactaaagggagtatcagcatcagtcgatgtggcaaccacagaaaatttggcaaatcttgtcacaattggaaaggcactcttgaaaaagccagtatccaggattaatttcgatacgggtagatatcaacctatccctaatggagggaccaatgaggaagccttaattaggtacttgatttaaataaatcattcataaagaatcacgctcattgcttgtcaataaaatatttatgtttatgtttaatactaatgcttgttttctaatacttttaacactttactttcttacatgagatgccgagacgagtgtagagtaatttattgtgtaggtaactttttgctctatatgagtcacttatataaaagtgacatatatatggtaataagttacctgtaagacgaggttaactatttgccataaataggtcactttacttatatagaagtgactcatttaagattaaaattaagttaccttttatttaaaattgacccatattgatttgaaaagtgacccatattgatttgaaaagtgacccatttaagctttaagtgaactgatgtgacaataaatttattatacacccggtgcacataatacaaattgtttaaattatcaagggtttgttggacaaaagtaattgttagttgtaagcttctagctatgagtttgtgagcttttagatgcctaggtagtttctaacttttagttatgaaactagttgtctaaagtgtttggtaataataattattgacgaaattttaacatgtaaataatatttaaatttggcaacttttgataaaagctaccgaaaagcttaatcatcttagattttgaccaagactactcaaaagctaaaagttatctaaaagttacatccaaaagctactttgaggaatatttaaacaattttttcaaagactaaaagctatcttaactacataaaaagtatgtcaaaagttacaccaaacatgtcctacattgaccacgttattctaacctacaaaactgactgggcaaacctgctactttgcaagaggtatcagtttattagggtgtttcatcttacctacctaaacagtaaaagtaaatatataaataaaacaaatattaattttatataaatattttatgagattagtattaatgtatatcctataatatcaacattcaaaaaacttttacgaatagataaaaagatatattaagaattaaaattatgcaaattcaaaagtcaattcaaattactcctattaaaaattggcggtatatgatttaaactttcaaaaataagaaaattataaaattatgtcactctttgttactactgaatacatgtttgtccaattgacaggtttgcgaaactccttaccgaggaaaagagcagacgcgaacaatatcggacgaaccgaagtgactaatatcacattttttaaacccatgtttcaatggatactatgattatatagtatatatatatgtatacaatacatcatgatctggaaaaaaacttacgctcgatttatgataaataaatttgtcaaaccatgtagctctcacaaaatctgtaatatttaatgaattttagtatgcgtagatatggcctatgggcgtggaatatttatccatgtaactcatttatttttacagctaagtcattgcattttaatctacgaaatttctcttttaatcaataacctaaaaataaatagtttgtgcatcaatttctctctatttactctgtaagtatttgttgtttttctttattgaacgataactacagtgccactcctatatatacaagagatcactttctaaacctagggataactatacaagaagagaaactaaccgttaaaatctttctacgatcaataaaaggaggaatatataatcacatgaaagtgcgaaataatcaatacaagtgagtttaattccctccgccactctaactcatttccctactctacacttaattctcccacgctatcaatcccattcatttactccagtatcagatgctagtaattcttcatagaatatgaaatatactaggattatattttgcgtttggatatagttttggtagaataacaattctactctagttacgttttctactattattgggatatcctttagaatgtaacctataaaatatgatcaataaaaacactcaaatcaaggaagtttacgcaaatatagcctggtatcaaagctatactaatcttaaagattattttttccttcgatcc

SEQ ID NO: 23 - DNA, 1224 bp, Artificial Sequence
  cDNA of Beta vulgaris phospholipase 1
atggagaattctagatctctgggtaaccctgttagccctagaccccctaatcatggtaatctcataacaattttaagtattgatgggggaggcattaggggaataatccctgcagttatgcttgaattccttgaatcacaactccagaagttagatggtgaggaagcaagattggctgattattttgatgttattgccggaacgagcaccggtggcctcataactgccatgttaaccgcccctaacgacaaaactcggccactctacgccgccaaggagattactcctttttatcttgagcattgtccgaagatcttccgccaaccaagtgggatatttggttcaatagggactctaatgaagctgctaagcgggccgaaatacgatggaaagtaccttcacaatctagtaaaggaattgctcggacaaagaaggttgcatcaagcgttgactaatgtggttatcccaacttttgatatcaagaatcttcagcctgttctcttttctacttatatggtcccaattgctaaagaattggacgtgttgctgtcagacatatgcataggcacgtctgcagctccaacgttcctaccagcgcatcattttgaaaacaaagatgatcagggcaatgtcaaagaattcaacctcattgatggtggtattgctgccaataatccttcattagtggcaataagcgaagtgacaaaacaaatagtgaagagcaacccgaatttcttcccgataaaggccacggatcgtgaacggttgctggtgatatcgttagggactggatccgacaaggtagagcagctctataatgctaaaagcgcagcaaagtggggaattatttcatggttatttgacaatggtaatactccactacttgatgcttttaatcaatcaaaggctgatatggtcgatttccacaattctgtggcctttcaagcatatggttctcttgacaattatcttcgcatccaagatgatacactaaagggagtatcagcatcagtcgatgtggcaaccacagaaaatttggcaaatcttgtcacaattggaaaggcactcttgaaaaagccagtatccaggattaatttcgatacgggtagatatcaacctatccctaatggagggaccaatgaggaagccttaattaggtttgcgaaactccttaccgaggaaaagagcagacgcgaacaatatcggacgaaccgaagtgactaa

SEQ ID NO: 24 - protein, 407 aa, Beta vulgaris
MENSRSLGNPVSPRPPNHGNLITILSIDGGGIRGIIPAVMLEFLESQLQKLDGEEARLADYFDVIAGTSTGGLITAMLTAPNDKTRPLYAAKEITPFYLEHCPKIFRQPSGIFGSIGTLMKLLSGPKYDGKYLHNLVKELLGQRRLHQALTNVVIPTFDIKNLQPVLFSTYMVPIAKELDVLLSDICIGTSAAPTFLPAHHFENKDDQGNVKEFNLIDGGIAANNPSLVAISEVTKQIVKSNPNFFPIKATDRERLLVISLGTGSDKVEQLYNAKSAAKWGIISWLFDNGNTPLLDAFNQSKADMVDFHNSVAFQAYGSLDNYLRIQDDTLKGVSASVDVATTENLANLVTIGKALLKKPVSRINFDTGRYQPIPNGGTNEEALIRFAKLLTEEKSRREQYRTNRSD

SEQ ID NO: 25 - DNA, 14701 bp, Beta vulgaris
  misc_feature (10783)..(10802): n is a, c, g, or t
gagtgtggagtagttgctttgtgcgagcgtgttttgtttgtgcgaacttctgctgtcacgttttgtttgtggaattgctgtcacgtttaattaccattcaagtgtgatctccttctagtagattgtgatcttgcttgtggtatattggatggtgtgagccccagacgtgattttgttcggttgatgcggttgtgcatcgtttctccaaaaccctagttggtttggtgcggttacgcatcgttattttgatgggttatggtggcccatccaagctattgtgttggtgcggttgtacatagttgatgccctaagtgacgaattgaatcatgaaggttggttggttgtccataattcaaaaagggtatttcttggttgtccataattcaaaaaaggtatttcttggttgtccctaatccaaaatggtgtgtattggttgtccctaatcttaaaagctggttattgaaggcgttgatttcacgtcttattggtctcctagtaataattcttttatatattttttcaattggagtgttggtgttactatcctatgattgaggggggagtattagagttatggtaagtatattatattagagtattatgtttggagtattatatttattaggagtcttgtattatatacctacgagctttcatatgcacgcgatgcgtgcgttaatttcaaaatttgttattctattagatactccattcgtactttatttatgattaaacttaaatgtgaaaaattcaacagttagatgaatttagatatattaattcgctaatgtaaaaaaataaaaaggttgtgagtgattgttaacattaattttttgtgaatgaatattgaacagaaagaacaaaaataatgagttggtttaactaaattaaatagtatcaaaagtagtgaatgttcagacttttcatgtgcacgttatgtatgccatcttttttttataagttataaatattttgtccatttaatttttgattgaagtatttgatgcatataccattttaaacttgttttaaatggcaagttggaatgagaattttttaaatgatttgcttttgtaattttttatattctattgattagatcattaagggtattttggtcactttaaaagaggacaccacacctcctcccttggcttatataatagagatctgttaagttgttagtacgtatatctagttcagtaaggatttctgatattaggttgtatatatatattcctcaaaagtttgataagtttcccatattctaaaccttaacactttgagtgagtgaaatgtggcagaagctaatttcttttatgtatattgatgatatacacagaatgcatgcatgtgtttatagaagacttaccattcaaaatcaacaatatacatggattagaacaatttttaaaatgtacttcaattttctctcactggacttggacacgattggggagaagaaggtggtggacaccgtgtaggaggagaagactgaagagaagacatacaccatacctttcaagaagaaggatagagtatgtgtgtatgtattagctaggcagactgttggagtctagaggttgagatgtggaataagaaggagaataatacgggtgagaggttttagttaattgtcaaatgttgcgctctagcatatgtccttattgatagatgactgtcaaagtttttgatcactagctccttatttcactactaaatactaattacactaatcgactgtacatacacccacacacatatatatacatatatgagaatgagggataacctagtggttaatgcttctctcccggttccaggagtcctatgatcgattctcacccttgacaagttaggttctcctttattccccaagcttatcacacgtacacacgtcgctgtcatagacatgtcatctttaagtttaagttaaaaatttataataaattaattaagtgtatggcatgcatgtatagttgcttccagcaattaattcctcctaaaattaaatagttagcttaccagtccacaatgtaggaataacaaagaataaatgggggaagtagagtgaatatattatataattcatataatagtctcgcggctattaagaagacgatttttgctaagctggttatggtgtgttgtttcttcttttttttctctcttgctcaggtaattaggttggtgtttgagaaataatactgaaaatgacgaacttacaaagctctcctccatccttcaattactacaacaggaagaaattggtcacaatccttagcatcgacggtggtggcattcgaggcattattcctgctgtcattcttgcttttcttgagcgacttcttcaggtacgtacataaaacataatcatactacatatacatatctcctatatatccattcatctctcgcactcatttgtactcatttagcgtgtgaatcgtgcatatcacatcgaacaatgttattttgatatgaataatgataattaggttcctagtagagttgggcatgatagccgggctagtccaacacgttccaccatgactttatccggttatccccacacgatacaattttgttcgaaagtgaaagacactgttatgggtcatatatagacatcatttttaaaatttggcataaatatgagaactatgtaatttctatcttgttatcattgataccttgtaaaactatgcaatcgtgcatgcacctaatgaataataacaataaacaataaagtaactaattaagtataatgagtagtgtacaattgtacatgtgcacaataatttcagatgcgaaatgaaaatattatttactacgttcataatatgttaaaaaaagcactcctgagacataatgtgatgcatagttaccccgcaaaaaacaattaattaatatgatgtcaggttaattggttataattatgtaggagttggatggagaggaagtaagactagcagattattttgatgtgatagcaggaacaagcacgggagggttgattacagccatgttaactgcaccagatgactataatcgtcctctatatgctgcgaaagatatcacaacattttacttgaagcatggtcctcaaatatttcctcaggaaaggtaaaaaatttaaatgtcagaatattccataccacaatataatttttaataagtagcctataaatggtggtcacacgctaagcatgacaattttattaaaagatcaatcgaatttttattaaatcttataggattaaaaattagaattcattgggtggaaaaaaaaatgaaaaaggttgtgatttttcgtccatcgttaaatcgaaacaaaaagaaaagtcaaagtaaaggcttattatttctcatttataaatatccaaattttagtacccaatacccataaatagttcgaaccatatagacacaataatcaattttcgtgtgaatggtttgtagggaaaccctatcctttcttatccataatggtgtataaataaattttacccacaaaaatatacaagtttcttcatatactatatcatgaaaataactattatgacatatatctacttagttacccgtcgagtaggtttactaaacttatccatacatcaaatatgtcaaaaagaatccagttaattgtttgaggatgtgagtcatgtgattggtgagctatcaattgttcatcactttctaaattcaaactcgaggaagtaatcaattggtcttggcatagtggttgtccactttgtcccttaatcaattatcgaggattcgattctcaatttttgggaatggaaagatatttttgaccagtcctttacccttaagtgtagcactcgaagcgagaggattaatcattgctgtcggcggtgaatacttagattgtttttaaaaaaaacttgagggagtgatactagcagatcatgtatcctcatgtttgtcaatgaaggtgtgcaaagtatatgctagtatgctactaccgcccatgaccctgaaattcaatttttcattgtttgttttagttgcattgtcctatttggctatttcaatactttagtaactttaaaaaaaaaatacttcctccatctctttttactcgctacactttttattatgggaagtttcacattacttgctacacttcttttttgggcaataaactatctctatctctctcctcccacatgagtcccgtgttgagatcctctagagttccaaaaaaactctacacggtagagttcgttaaatatcagtcgttgattaagaaatcaaaggcttgtattttgttttccaaaaatcccccctattttcccccgaatatcctgccaatatcttttccttttccaccaatcatgagcctttgattttatgatatatggtcaggattcaactctactttgtagagttttcataaaactctagaggatccggaccccatgagtcccttttctttttattctctacttctctcttctccaaaaattgcctaggagtccgtgaaatgagaagtgtagcgagtaaaaagaaacggatgaagtatattgttaatattttttaaaatatatatattttattgtaggattaatcttaataattactaagggatttccaacatgtttgatgtcgcctgtattttgctgaccaagtttagaaaaattgataggttgtttctaacatctttttgccggccaccaagctggagatgtagacatatagaagtagtttatgattttcccactttgaactggttatacatacattaattagttattacaagtcttttttagatgattactccatcgattccaccattgttcatgtcatcttgtcatatacagcgactttcgtaactattgtgtattattattatatactccctctttaccaatctagatgcaattattttccttttatggtttctccggacacactttttacatctatgattatatattagtagaatttagttatagatgatatattgtaaatttatacattattgaaacaaatctaatatgatatttatatgataattttatttgcttatatcagtaaaaaaatatgcttagttaacattgatgatctttaaccctagaaaaacaaatgttgcaagttatatggaattaacaaaggaggttatatttttcttggaaaagaaccatagttgtctctttccttgaagtacaattatgatgtcagtgggtaatggaatctacccggatccaaatcattttttagcgatttgtatcctcaaattttggacccaacggatatggatcatgtcttaaatcattacatggagtcgtatccatttacccattttttaaaaattattttaaaatatataattaaaagtgaaaaacttaaaggattttttaactggaataatacaaactttgggccgttctctcgcaataatacaaacttttgattattttttaataatacaaactttaggccaaaattcctccagtaggttaataccggttggtaacttgttgtaggaggtaaccaagctgacgtggcacctttaggacacgtgtctttatttgattggctgtttttttaaatttagggaaaaaaaaaaccaaaatttttcttttttttttctttcttctcctgctccccccttcattctctttctcactactccaccccaccgacccccacccctggcccctgcccccagcccctccctgcctgcacaccgcatccctccgacgaccaaccccccatctctggcccttcccccaccccgaaaccataccgcacccctccgacaaccacccctggcccctcccccacccgaaaaccacaccgcacctcttcgacaaccaacccccatttctggcccctcccccaccccgaaaccacactgcacccctccaacggccatcacctgacgccattctcgatcgctcgaacttagatcctttcccgcacaacaacaagtcgtcgtcgtcaccgcgcgaaatcaatacgatattcgaaaatggcggtcattttattatcgacgaattggaggaggaggaagagacgtcgttgttgacgatttcgcatagttacgcgatctggggaagtggtttcgtgtggtggtgagtttgaggtggtttcgtggtgggggagtttgaggcggtttcatggttggggacgaggtggtgatggtggtttcatccgtgggggtggagctgtgggagggggtggaactgtggaggtgagggtggggggagggggtgggggtggagctgtggaggtgggggaagggggtgggagtggagccgtggaggtggaggagggggtgggagtgggctttcacattttcagttggttggctaggggaaggaggaagagattttggagtttaaaaaaatcgacctattctacatgttaatggtcaacttgacctactggaggaattttggcctaaagtttgtattattaaaaaataatcaaaagtttgtattattgcgagagaacggcccaaagtttgtattattcgagttaaaaaatccaaacttaaaaccattttatgattttatctttcaaattacttatatgtttattgtgatgaatatttatgttgtcattattattctttgtaatgtacaaatatgattttgcaatgaacaacatactatcatatacttcctccatttctaaataagtgcaacatttcttgttttcacatttgccaatgcattattttaaccagtaatatcttcaattatcaataagtaaaaattataaaaagttgatattaaaaaaattcacatttagatgaatctaacaagatcccacatgactatgtttttcctaaaatgcaaatcactaaagctaattgatgtttaaactgtgaatagtaaacactatgcaaatgttacacttatttagaaacggaggaagtaataaataacccaattgaatagttatataattatcaaaaaataagtaattacaaaagatggttaattcataatgtagtatgtacccaagtgtagaaatataaccaaaataatataatatatttctaattaaacactattgagttcattaagaagatattcttgcttttgagcttccttccatttccgattgatttgaatagtgagatctcgacaccataacgtatcttagttgtttgaactagtcgaattgaactgatacaagaaaggaaatagcagtagttaaaaaaaattattcaagtttataatacaatgaacataatttttcaaacatacaattaacacattctaataatacaataaacatgctcccgcacatagtcccgactattaggctgtgcaaacaacccaatagcacaggaccccgaatttcttagggtccccaaaatctggaaacaaaaaaatatagttgattacggcgctaaaacaattcaactacatatattagcagagttgttatatgagattaactctacaacaagaatacgcaagttcgactcatgttccgggaatatctttacatactttttgcaagtgtttatgatattttcttctagtttgagcatttcactcatctccccaccacttcatacttactttctaactattttccttacttttttttcaatacttttttttgataaattgtttttctcaattctttagggtacttttttgataaattcttttatcaattccttagggtacttattttttttggaagtgtatatttgtccaataagaattgaataatttcctgccacaagtttactagtttaccggtttagtcacctcatcatatatataaatttttttttttttgttgtaccttttagagtgagatagaaaaattattatcgttatctttataagtagaacatcagtcataatgtggttttatattgagttgttacacacaatttcaaatgagtttgaggttttagtttttcgatttacaagataaatttatataattgtaatattataaaagattttttttatcatttgagttgcaaaaaaatgagattaggggtccaatcctaaaattggaacaagacctccaaaatgtttaagacggccctgcccgcacacaatgagcatgtgattaaaatgagcatgttagtaatacaatgaacatcaacctaaaaatgtgcaccttgtatttgtaaatggtacaataaatatcacataatcatacaaagaacatttgaacaaatatcacacatttatagacaaatatatatgataatcaacccatcattaattcatatcatttcattgaatatattacaaacacataacgaattatgactgaaatgcaataaacatctgaccaacatgtgtttcagtgaacatattctgattggacaatgaacatatgccataattcatgttattaatgcaattaatatgtgtcaaagacataataaatatatgaagaactgtacataacatctgaacaaacacataataaacatatggctaaatgtaataaacatatgaccaacacaaattcaattagtacattacaataatacaacgaacatatatttacagtacaacattacctgtttttttctagatgtcgaactcgttcatctcctttattcattgggctctctcatttgttcattgggacatcaattgcaaggttgttttcatttttcacaaatatcaagatcttcactagaaaagatggaaaaaaaaataagaaatgaaagtgcaatatgtaaaaaaaaatattcttttttcttatcaaatgcatagatctaataacttatgttctttgcaactcgttgtattcatcttcatgtacgaaaattgtttaaaaaaatgaagaatttaaaaaggttgatgagaaaggttagagagaagttaaagagatgttggaggatttggggagaagagataaaaagtctttgaaaatttctggggaaaaatgaaagtaatgaattcaaatttttttatgttttttggtgttcattggagatcaacaaatgttcatttcgtgcatttttggtttaatgaatacgcgttttatgttttgttgacatccgttttgacccatgcacaccttcctcaacatacatccgttcgcacggttgatctactgatcattcgcttgaaaagggaataaggtcatgacagcgttaagaatgaaacaagaaagatcgtatatttgttggtaacttggtactacaattagggttgttcaccggtccaggatcggatcgaacctgacctgcctggaccgttctttatgggattcttcggaccaggtgtggatcggaaaaatcaggtctggtcttcagtccggacctgttgggccggaaaaattaacttgtatctctgattcttcggacctgttacgacccaccatcaataaatatcagaattccatagatttatcagtttacagaggaccaactacaacaagcaaacaaaaaaacaattctagtacttcctccgtttttttttttacttgcaacacttttttttcatcaactccaatgtaaaatttgggtatgagataggcatacaggaaaaaaagagagatccccatgtgattggagagagatagagagaaaggaaaagaaaaagtagaaagtgttgcaagtaattaattattttctttttaggaaagtgttgcaagtaaaaagacggaggaagtatttagtttttattacaaattgtttggggggggggggcaggagacatggagtcacactagactaggacactcaaagaggcaccaatgctactcactaagtgattaaagttaaagatagaaaagggtgaaaaagactcgcgaactgaaaaacaaacctgatcggtggtgggcggtagctgcggtcgcctgagcggcgtcgtggcgtcggtgcgactggtttggcgaggcgtgaccgcgtgaggactgaggtgtttgagttctcttagggtttcttttagaatgactaaatgagagagggagaagtaggaataaagggctggcatttttttaaaaaaaaaaaatactaaaaagcttccgagttttcggtctggaccggattttttcgagtttgaaccagaccgaaccggaaacccggaatagacacattccacggaccggggaccggattggaatcgccggtccggttcgatccgatccaaaatccggtccgattagatccgacccacctatgtgaacagccctagctacaatactacatgactacctgccttattaactctcccttttattagatttttcgttagctaataactcccttaggatattgaatctactttgttggttataactcttataagttactattatagtaggagaacaactattattatgtgcaaaattacacagaatttgtttttcttccatttttaggggaccacttgctcagctgattagcttcatcaaagcaatgacagggccaaaatatgatggcaagtatttacgccatatactaagggaaaaattgaaagagacaaggttgcatcacacactaacaaatgttgtcattccaacttttgacattaagaccttccaaccagttatattctcttcctacaaggtaaataaattataatcgtgtgctcatctccaataattttaccttaaatgaattttcatcaactaatcatttgctttgctgatgaccatccttgatttgaatgaagagaatatatatatatatatatatatatatatatatatatatatatatatatatatatattatatatactatatatatagtacgtagtacgtacgtacgttacgtacgttacgtagtacgtacgggtacttaacgtcgtannnnnnnnnnnnnnnnnnnnagtatagtagtatatatatatatatatatatatatatatatatatatatatatatatatatatatatatatatatatatatatatatatatataggatgaggaactagctcatgtggtagagcactcccctctgatccttgaggtcaggggttcgatccttacccccaacattatgttggggcatttccttagcatgctttgcatgctttaccagccaatgtgctggtagttcctacaaggctagtagaatgaattttacgtgttataactcatatgaataagtgatgtaactccaaaaaaaaaaatattagaaaaaagaaattcaagaaaaaaaaaattgggatcaaaattttttaaggggtataactctaataaagtattgtaactctaatccaatcatgtggtcgaaattcattctcatttctcatttaaagagcattctcatatgatattactcctatatatattcgtgcttgtttttttctttattagatgatcctagcttgatatcgacgcaaactaagaacttcaaaaggaaataatgaaattactattttaatgttttctttttgttttattccatatatatgtaaacacagtattatcgatctgataggcataaatgttatacttaatgtgattatccaaatagtttaattgagagttttactcttatcaagttatcatgtcgtctagtgttaataattctttagttttatgtctattttgtcgtagctatagtccgactggtcaagtacttgatcaaacagtttaagcggtgaacctattgcatgacttttacctaggcaactagtatatgtctggaaaagtgaatgacgatctctcattttcatagtgaaatttacaatattctctaagcttttatgatattaatgataggtgatatatgatgcgaggttattgaagtgtgtggattttcctagtgccctttagttacattgttaatttgttagggttgattcaagtagatttacagacctatatgagggcataactaagagaccatattttattgatggaagaaaagtagagagggtcactttagcagctactcctactacgagtagctaagtattacggatttaaaaaatattcctcccaatgatagaaattaaggtcgaaataaaacaacattttaagataacacatatttataaaaacaaaactagtgaaaaataacctagacaaattcgaatcttatttgcatcgacaaactccaacattttcatcattattttcaaaaacatatcaaaacattgaaaatgccagatcttctgtccgccccctccctttgaccaaaatatgaatttatacgtaagtagttttaccttcgtaattttacatttgtgattttgtagacttcaattaacattttcatttgtgttcaattaaactttgcgacttagtcaacggattaattacatccttctttatgcataaaaaagtccatttatcaatcaacccaagaagactcacaatgtttttatcatttaatttttgcaaattctaagttatcatttaatttttacagattctaagttatcctgatctggatgcgaaattatcagatatatgtataggcacatcggccgctcctaccattctgccttctttctatttccaaaatgcatttgaaaacgaaaagacaagggaattcaacctcattgatggtggaattgtgagtacaaatccggtaagtcaagctcaatcaatcatattattattcttatgcttagaggatgcacaatagcatggtttcacttggggcaaaggtgaaccaatgggtgaggttggtcttaccattggggtgagtcaaggcaaacatggcttaatgaggttgggataatttgctccccctctctcccaacccatgcatcggaccaagagcccaagctagtaacaaaaggcttgtgtactttcacagagaatgagcttcatgtctttgagtgtagagcttttttccttcccaaacgtcctactcttagaattgttatttacataacctactttaattatttttttttattaatttataaaatagttgttatgttattacatagtaagttgtcgtatcagagttcttttcacgaaaactcaaagctgaaacataaaaacagacgagtttattcatcataccacctagatataccacaatgttagtacattttgttaatttggaactatccaaatgaacaataagcagaaaaatagtcttgagtgtaatgtctacaatgttcacaatacattcaagtgtatgttgaattttttgtataagagcctaaaaaacttttatccaacaatactttaaaccagcagatagaatattatttgatgtatcaataatttcattctatctttttgttttgtcgtctgggcagacttatctggcaataaatgaagttaccaaacaaatgatgaaggagaatccagattacgggaccatccataataagttgctggttttatcgataggaacaggatcaggaaaaattgagcagaaatacaatgctaaaactgcaggaaagtgggggcttgtctcttggctttttcaaaatggatcatcaccaattataagtgctttttatgaagccggggctgacttagttgattaccaaaataatatcctcttccaatcgtttcgttcagaggacaagtaccttcgtgtgcaagtaagtcgcatgatacccttcaaatttaactttaatgtagtaatccgtttacgattaatcggcacatattgttggaaataaaacaggatgacagcttaacaggaacaactgcttcaacagatgtagcaacagagaagaacttggaaaatctagtgaaaattggtcaagaattgcttaacaaaccagccagcagggtggacccagaaactgggcatctgaaagcaattccacaccttggtaccaatgcagatgctcttcgaaggttggttcataaattttataatattgccaatataaattgcacattattagttattactactagatagattaacaagtcattaacaaataggttcgcaaaacaactctcggatgaaagaaaataccgcaggggcaaagactccaatcagatgcaagagtacagctgagctgacgatgtgcaggcatttctgagtactgagctgtctttgattgtatactatatgataaatgtgtgcaatgtaattgacctcaaatcttctatctcataatttttgtactattctgttggttgattataaatttgtaacgttctaaagattatcttaaaaggtactagaccgtagtacaatacctgctaataatatatagtagcatacattctttttttggctcccttccgggaatccgtggtaagatgaatttcctttagactgtcctcacacagggccactcacccagaagaccaacaacccccctccccccaactatattgaaatttttgcttgcaccaagatttgaaccttggcttcccatatgtgagacacgaaaccataccattggacccaagggtccttggtatataaagtagcatacatgtgacacacaaagagagacagtagatgttgcttcaggtaatgcagaaaccccctatatgatcaacatgatcaacagaactatgtatatctatacttctttccctagataagcaagaatttatggaggctaactatccttgtttccctgtaatgcttatacaagaagatgcaaaatagaaagctcagagccagatactctcttaatagacccaggagtaacctgaacttgctaccatattcaacacatttaagccagaaggtaaaacacagaagttcgaaagtaaagacagcaagttcacaaagctagggatctttttgaagtgcaaccatcggacattatgggattgctaa

SEQ ID NO: 26 - DNA, 1215 bp, Artificial Sequence
  cDNA of Beta vulgaris phospholipase 2
atgacgaacttacaaagctctcctccatccttcaattactacaacaggaagaaattggtcacaatccttagcatcgacggtggtggcattcgaggcattattcctgctgtcattcttgcttttcttgagcgacttcttcaggagttggatggagaggaagtaagactagcagattattttgatgtgatagcaggaacaagcacgggagggttgattacagccatgttaactgcaccagatgactataatcgtcctctatatgctgcgaaagatatcacaacattttacttgaagcatggtcctcaaatatttcctcaggaaaggggaccacttgctcagctgattagcttcatcaaagcaatgacagggccaaaatatgatggcaagtatttacgccatatactaagggaaaaattgaaagagacaaggttgcatcacacactaacaaatgttgtcattccaacttttgacattaagaccttccaaccagttatattctcttcctacaagattctaagttatcctgatctggatgcgaaattatcagatatatgtataggcacatcggccgctcctaccattctgccttctttctatttccaaaatgcatttgaaaacgaaaagacaagggaattcaacctcattgatggtggaattgtgagtacaaatccgacttatctggcaataaatgaagttaccaaacaaatgatgaaggagaatccagattacgggaccatccataataagttgctggttttatcgataggaacaggatcaggaaaaattgagcagaaatacaatgctaaaactgcaggaaagtgggggcttgtctcttggctttttcaaaatggatcatcaccaattataagtgctttttatgaagccggggctgacttagttgattaccaaaataatatcctcttccaatcgtttcgttcagaggacaagtaccttcgtgtgcaagatgacagcttaacaggaacaactgcttcaacagatgtagcaacagagaagaacttggaaaatctagtgaaaattggtcaagaattgcttaacaaaccagccagcagggtggacccagaaactgggcatctgaaagcaattccacaccttggtaccaatgcagatgctcttcgaaggttcgcaaaacaactctcggatgaaagaaaataccgcaggggcaaagactccaatcagatgcaagagtacagctga

SEQ ID NO: 27 - protein, 404 aa, Beta vulgaris
MTNLQSSPPSFNYYNRKKLVTILSIDGGGIRGIIPAVILAFLERLLQELDGEEVRLADYFDVIAGTSTGGLITAMLTAPDDYNRPLYAAKDITTFYLKHGPQIFPQERGPLAQLISFIKAMTGPKYDGKYLRHILREKLKETRLHHTLTNVVIPTFDIKTFQPVIFSSYKILSYPDLDAKLSDICIGTSAAPTILPSFYFQNAFENEKTREFNLIDGGIVSTNPTYLAINEVTKQMMKENPDYGTIHNKLLVLSIGTGSGKIEQKYNAKTAGKWGLVSWLFQNGSSPIISAFYEAGADLVDYQNNILFQSFRSEDKYLRVQDDSLTGTTASTDVATEKNLENLVKIGQELLNKPASRVDPETGHLKAIPHLGTNADALRRFAKQLSDERKYRRGKDSNQMQEYS

SEQ ID NO: 28 - DNA, 40 bp, Artificial Sequence
  R59Q mutant - primer AlleleX
gaaggtgaccaagttcatgctccgtccagctcctgcagct

SEQ ID NO: 29 - DNA, 39 bp, Artificial Sequence
  R59Q mutant - primer alleleY
gaaggtcggagtcaacggattcgtccagctcctgcagcc

SEQ ID NO: 30 - DNA, 22 bp, Artificial Sequence
  R59Q mutant - primer common
tccccggaaccatccttgcctt

SEQ ID NO: 31 - DNA, 201 bp, Artificial Sequence
  partial sequence indicating detectable single nucleotide polymorphism that causes amino acid substitution R59Q in Sorghum bicolor phospholipase
gagcccgtcgtgctggggcagagggtgacggtgctgacggtggacggcggcggcatccgtggtctcatccccggaaccatccttgccttcctcgaggcccrgctgcaggagctggacgggccggaggttaggctcgcggactacttcgactacatcgccgggacgagcaccggcgggctcatcaccgccatgctcaccgcg

SEQ ID NO: 32 - DNA, 41 bp, Artificial Sequence
  V162I mutant - primer AlleleX
gaaggtgaccaagttcatgctgagcgacacgctcaccaaca

SEQ ID NO: 33 - DNA, 41 bp, Artificial Sequence
  V162I mutant - primer AlleleY
gaaggtcggagtcaacggattgagcgacacgctcaccaacg

SEQ ID NO: 34 - DNA, 21 bp, Artificial Sequence
  V162I mutant - primer common
ctgcagcagcctgacgtcgaa

SEQ ID NO: 35 - DNA, 201 bp, Artificial Sequence
  partial sequence indicating detectable single nucleotide polymorphism that causes amino acid substitution V162I in Sorghum bicolor phospholipase
catgtccgcgctgaggaagccaaggtacaacggcaagtgcctccgtaacctgatcatgagcatgctcggcgagacgagggtgagcgacacgctcaccaacrtcatcatccctaccttcgacgtcaggctgctgcagcccatcatcttctccacctacgacgtacgtacgccgccggccgccgtcgtcatgaataatcaatc

SEQ ID NO: 36 - DNA, 39 bp, Artificial Sequence
  S291L mutant - primer AlleleX
gaaggtgaccaagttcatgctggcagatgccccaccgcg

SEQ ID NO: 37 - DNA, 39 bp, Artificial Sequence
  S291L mutant - primer AlleleY
gaaggtcggagtcaacggattggcagatgccccaccgca

SEQ ID NO: 38 - DNA, 19 bp, Artificial Sequence
  S291L mutant - primer common
gcctgtacacggcgcggca

SEQ ID NO: 39 - DNA, 201 bp, Artificial Sequence
  partial sequence indicating detectable single nucleotide polymorphism that causes amino acid substitution S291L in Sorghum bicolor phospholipase
ctgtacccagtgaagccgtggaactgccgcaagttcctggtgctgtccatcgggacggggtcgacgtcggagcagggcctgtacacggcgcggcagtgctygcggtggggcatctgccggtggatccggaacaacggcatggcccccatcatcgacatcttcatggcggcgagctcggacctggtggacatccacgtcgcc

SEQ ID NO: 40 - DNA, 39 bp, Artificial Sequence
  Q372stop mutant - primer AlleleX
gaaggtgaccaagttcatgctgaccctggacacccgctg

SEQ ID NO: 41 - DNA, 42 bp, Artificial Sequence
  Q372stop mutant - primer AlleleY
gaaggtcggagtcaacggattgttgaccctggacacccgcta

SEQ ID NO: 42 - DNA, 20 bp, Artificial Sequence
  Q372stop mutant - primer common
gtcgggatcggggagcggat

SEQ ID NO: 43 - DNA, 197 bp, Artificial Sequence
  partial sequence indicating detectable single nucleotide polymorphism that causes amino acid substitution Q372stop in Sorghum bicolor phospholipase
gcatccaggacaactcgctgcacggcgccgcggccaccgtggacgcggcgacgccggagaacatgcggacgctcgtcgggatcggggagcggatgctggcgyagcgggtgtccagggtcaacgtggagacagggaggtacgaaccggtgcctggggaaggaagcaacgctgatgcgctcgctgggatcgcaaggcag

SEQ ID NO: 44 - DNA, 19 bp, Artificial Sequence
  Forward Primer
ggcccccatcatcgacatc

SEQ ID NO: 45 - DNA, 24 bp, Artificial Sequence
  Reverse Primer
aatcaggcaacaaattcacttctc